European Patent Application EP 4 512 255 A1, published February 26, 2025. Title: Anti-human coronavirus composition. Applicant: Meiji Co., Ltd. Application JP, filed April 19, 2023. The sequence listing filed with the application follows.

SEQUENCE LISTING (1 sequence)

SEQ ID NO: 1 - RNA, 502 nt, Lactobacillus delbrueckii subsp. bulgaricus OLL 1073 R-1
  source 1..502: mol_type = rRNA
gctggcggcgtgcctaatacatgcaagtcgagcgagctgaattcaaagatyccttcgggrtgatttgttggacgctagcggcggatgggtgagtaacacgtgggcaatctgccctaaagactgggataccacttggaaacaggtgctaataccggataacaacatgaatcgcatgattcaagtttgaaaggcggcgyaagctgtcactttaggatgagcccgcggcgcattagctagttggtggggtaaaggcctaccaaggcaatgatgcgtagccgagttgagagactgatcggccacattgggactgagacacggcccaaactcctacgggaggcagcagtagggaatcttccacaatggacgcaagtctgatggagcaacgccgcgtgagtgaagaaggttttcggatcgtaaagctctgttgttggtgaagaaggatagaggcagtaactggtctttatttgacggtaatcaaccagaaagtcacggctaactacgt